European Patent Application EP 4 520 829 A1, published March 12, 2025. Title: METHOD FOR PRODUCING AMINO ACID AND PEPTIDE COMPOUND USING ENZYME AND ADDITIVE. Applicant: CHUGAI SEIYAKU KABUSHIKI KAISHA. Application JP. The sequence listing filed with the application follows.

SEQUENCE LISTING (21 sequences)

SEQ ID NO: 1 - protein, 332 aa, Pseudomonas putida KT2440
MRVPFTELQSLLQAIFQRHGCSEAVARVLAHNCASAQRDGAHSHGVFRMPGYVSTLASGWVDGQATPQVSDVAAGYVRVDAAGGFAQPALAAARELLVAKARSAGIAVLAIHNSHHFAALWPDVEPFAEEGLVALSVVNSMTCVVPHGARKPLFGTNPIAFAAPCAEHDPIVFDMATSAMAHGDVQIAARAGQQLPEGMGVDADGQPTTDPKAILEGGALLPFGGHKGSALSMMVELLAAALTGGHFSWEFDWSGHPGAKTPWTGQLIIVIDPGKAEGQRFAQRSRELVEHMQAVGLTRMPGERRYREREVAEEEGVAVTEQELKGLKELLG

SEQ ID NO: 2 - protein, 332 aa, synthetic construct
  REGION 1..332: note = H44X
  VARIANT 44: note = A, R, N, D, C, Q, E, G, I, L, K, M, F, P, S, T, W, Y or V
MRVPFTELQSLLQAIFQRHGCSEAVARVLAHNCASAQRDGAHSXGVFRMPGYVSTLASGWVDGQATPQVSDVAAGYVRVDAAGGFAQPALAAARELLVAKARSAGIAVLAIHNSHHFAALWPDVEPFAEEGLVALSVVNSMTCVVPHGARKPLFGTNPIAFAAPCAEHDPIVFDMATSAMAHGDVQIAARAGQQLPEGMGVDADGQPTTDPKAILEGGALLPFGGHKGSALSMMVELLAAALTGGHFSWEFDWSGHPGAKTPWTGQLIIVIDPGKAEGQRFAQRSRELVEHMQAVGLTRMPGERRYREREVAEEEGVAVTEQELKGLKELLG

SEQ ID NO: 3 - protein, 332 aa, synthetic construct
  REGION 1..332: note = F117X
  VARIANT 117: note = A, R, N, D, C, Q, E, G, H, I, L, K, M, P, S, T, W, Y or V
MRVPFTELQSLLQAIFQRHGCSEAVARVLAHNCASAQRDGAHSHGVFRMPGYVSTLASGWVDGQATPQVSDVAAGYVRVDAAGGFAQPALAAARELLVAKARSAGIAVLAIHNSHHXAALWPDVEPFAEEGLVALSVVNSMTCVVPHGARKPLFGTNPIAFAAPCAEHDPIVFDMATSAMAHGDVQIAARAGQQLPEGMGVDADGQPTTDPKAILEGGALLPFGGHKGSALSMMVELLAAALTGGHFSWEFDWSGHPGAKTPWTGQLIIVIDPGKAEGQRFAQRSRELVEHMQAVGLTRMPGERRYREREVAEEEGVAVTEQELKGLKELLG

SEQ ID NO: 4 - protein, 332 aa, synthetic construct
  REGION 1..332: note = M141X
  VARIANT 141: note = A, R, N, D, C, Q, E, G, H, I, L, K, F, P, S, T, W, Y or V
MRVPFTELQSLLQAIFQRHGCSEAVARVLAHNCASAQRDGAHSHGVFRMPGYVSTLASGWVDGQATPQVSDVAAGYVRVDAAGGFAQPALAAARELLVAKARSAGIAVLAIHNSHHFAALWPDVEPFAEEGLVALSVVNSXTCVVPHGARKPLFGTNPIAFAAPCAEHDPIVFDMATSAMAHGDVQIAARAGQQLPEGMGVDADGQPTTDPKAILEGGALLPFGGHKGSALSMMVELLAAALTGGHFSWEFDWSGHPGAKTPWTGQLIIVIDPGKAEGQRFAQRSRELVEHMQAVGLTRMPGERRYREREVAEEEGVAVTEQELKGLKELLG

SEQ ID NO: 5 - protein, 332 aa, synthetic construct
  REGION 1..332: note = T156X
  VARIANT 156: note = A, R, N, D, C, Q, E, G, H, I, L, K, M, F, P, S, W, Y or V
MRVPFTELQSLLQAIFQRHGCSEAVARVLAHNCASAQRDGAHSHGVFRMPGYVSTLASGWVDGQATPQVSDVAAGYVRVDAAGGFAQPALAAARELLVAKARSAGIAVLAIHNSHHFAALWPDVEPFAEEGLVALSVVNSMTCVVPHGARKPLFGXNPIAFAAPCAEHDPIVFDMATSAMAHGDVQIAARAGQQLPEGMGVDADGQPTTDPKAILEGGALLPFGGHKGSALSMMVELLAAALTGGHFSWEFDWSGHPGAKTPWTGQLIIVIDPGKAEGQRFAQRSRELVEHMQAVGLTRMPGERRYREREVAEEEGVAVTEQELKGLKELLG

SEQ ID NO: 6 - protein, 332 aa, synthetic construct
  REGION 1..332: note = H182X
  VARIANT 182: note = A, R, N, D, C, Q, E, G, I, L, K, M, F, P, S, T, W, Y or V
MRVPFTELQSLLQAIFQRHGCSEAVARVLAHNCASAQRDGAHSHGVFRMPGYVSTLASGWVDGQATPQVSDVAAGYVRVDAAGGFAQPALAAARELLVAKARSAGIAVLAIHNSHHFAALWPDVEPFAEEGLVALSVVNSMTCVVPHGARKPLFGTNPIAFAAPCAEHDPIVFDMATSAMAXGDVQIAARAGQQLPEGMGVDADGQPTTDPKAILEGGALLPFGGHKGSALSMMVELLAAALTGGHFSWEFDWSGHPGAKTPWTGQLIIVIDPGKAEGQRFAQRSRELVEHMQAVGLTRMPGERRYREREVAEEEGVAVTEQELKGLKELLG

SEQ ID NO: 7 - protein, 332 aa, synthetic construct
  REGION 1..332: note = Q186X
  VARIANT 186: note = A, R, N, D, C, E, G, H, I, L, K, M, F, P, S, T, W, Y or V
MRVPFTELQSLLQAIFQRHGCSEAVARVLAHNCASAQRDGAHSHGVFRMPGYVSTLASGWVDGQATPQVSDVAAGYVRVDAAGGFAQPALAAARELLVAKARSAGIAVLAIHNSHHFAALWPDVEPFAEEGLVALSVVNSMTCVVPHGARKPLFGTNPIAFAAPCAEHDPIVFDMATSAMAHGDVXIAARAGQQLPEGMGVDADGQPTTDPKAILEGGALLPFGGHKGSALSMMVELLAAALTGGHFSWEFDWSGHPGAKTPWTGQLIIVIDPGKAEGQRFAQRSRELVEHMQAVGLTRMPGERRYREREVAEEEGVAVTEQELKGLKELLG

SEQ ID NO: 8 - protein, 332 aa, synthetic construct
  REGION 1..332: note = W253X
  VARIANT 253: note = A, R, N, D, C, Q, E, G, H, I, L, K, M, F, P, S, T, Y or V
MRVPFTELQSLLQAIFQRHGCSEAVARVLAHNCASAQRDGAHSHGVFRMPGYVSTLASGWVDGQATPQVSDVAAGYVRVDAAGGFAQPALAAARELLVAKARSAGIAVLAIHNSHHFAALWPDVEPFAEEGLVALSVVNSMTCVVPHGARKPLFGTNPIAFAAPCAEHDPIVFDMATSAMAHGDVQIAARAGQQLPEGMGVDADGQPTTDPKAILEGGALLPFGGHKGSALSMMVELLAAALTGGHFSWEFDXSGHPGAKTPWTGQLIIVIDPGKAEGQRFAQRSRELVEHMQAVGLTRMPGERRYREREVAEEEGVAVTEQELKGLKELLG

SEQ ID NO: 9 - protein, 332 aa, synthetic construct
  REGION 1..332: note = K260X
  VARIANT 260: note = A, R, N, D, C, Q, E, G, H, I, L, M, F, P, S, T, W, Y or V
MRVPFTELQSLLQAIFQRHGCSEAVARVLAHNCASAQRDGAHSHGVFRMPGYVSTLASGWVDGQATPQVSDVAAGYVRVDAAGGFAQPALAAARELLVAKARSAGIAVLAIHNSHHFAALWPDVEPFAEEGLVALSVVNSMTCVVPHGARKPLFGTNPIAFAAPCAEHDPIVFDMATSAMAHGDVQIAARAGQQLPEGMGVDADGQPTTDPKAILEGGALLPFGGHKGSALSMMVELLAAALTGGHFSWEFDWSGHPGAXTPWTGQLIIVIDPGKAEGQRFAQRSRELVEHMQAVGLTRMPGERRYREREVAEEEGVAVTEQELKGLKELLG

SEQ ID NO: 10 - protein, 342 aa, synthetic construct
  REGION 1..342: note = wild type NMAADH-linker-His tag
MRVPFTELQSLLQAIFQRHGCSEAVARVLAHNCASAQRDGAHSHGVFRMPGYVSTLASGWVDGQATPQVSDVAAGYVRVDAAGGFAQPALAAARELLVAKARSAGIAVLAIHNSHHFAALWPDVEPFAEEGLVALSVVNSMTCVVPHGARKPLFGTNPIAFAAPCAEHDPIVFDMATSAMAHGDVQIAARAGQQLPEGMGVDADGQPTTDPKAILEGGALLPFGGHKGSALSMMVELLAAALTGGHFSWEFDWSGHPGAKTPWTGQLIIVIDPGKAEGQRFAQRSRELVEHMQAVGLTRMPGERRYREREVAEEEGVAVTEQELKGLKELLGGGSSHHHHHH

SEQ ID NO: 11 - protein, 375 aa, synthetic construct
  REGION 1..375: note = W253H-SBP tag-linker-His tag
MRVPFTELQSLLQAIFQRHGCSEAVARVLAHNCASAQRDGAHSHGVFRMPGYVSTLASGWVDGQATPQVSDVAAGYVRVDAAGGFAQPALAAARELLVAKARSAGIAVLAIHNSHHFAALWPDVEPFAEEGLVALSVVNSMTCVVPHGARKPLFGTNPIAFAAPCAEHDPIVFDMATSAMAHGDVQIAARAGQQLPEGMGVDADGQPTTDPKAILEGGALLPFGGHKGSALSMMVELLAAALTGGHFSWEFDHSGHPGAKTPWTGQLIIVIDPGKAEGQRFAQRSRELVEHMQAVGLTRMPGERRYREREVAEEEGVAVTEQELKGLKELLGGTDEKTTGWRGGHVVEGLAGELEQLRARLEHHPQGGSHHHHHH

SEQ ID NO: 12 - protein, 6 aa, synthetic construct
  REGION 1..6: note = His tag
HHHHHH

SEQ ID NO: 13 - protein, 34 aa, synthetic construct
  REGION 1..34: note = SBP tag
GTDEKTTGWRGGHVVEGLAGELEQLRARLEHHPQ

SEQ ID NO: 14 - protein, 332 aa, synthetic construct
MRVPFTELQSLLQAIFQRHGCSEAVARVLAHNCASAQRDGAHSHGVFRMPGYVSTLASGWVDGQATPQVSDVAAGYVRVDAAGGFAQPALAAARELLVAKARSAGIAVLAIHNSHHFAALWPDVEPFAEEGLVALSVVNSVTCVVPHGARKPLFGTNPIAFAAPCAEHDPIVFDMATSAMAHGDVQIAARAGQQLPEGMGVDADGQPTTDPKAILEGGALLPFGGHKGSALSMMVELLAAALTGGHFSWEFDQSGHPGAETPWTGQLIIVIDPGKAEGQRFAQRSRELVEHMQAVGLTRMPGERRYREREVAEEEGVAVTEQELKGLKELLG

SEQ ID NO: 15 - protein, 332 aa, synthetic construct
MRVPFTELQSLLQAIFQRHGCSEAVARVLAHNCASAQRDGAHSHGVFRMPGYVSTLASGWVDGQATPQVSDVAAGYVRVDAAGGFAQPALAAARELLVAKARSAGIAVLAIHNSHHFAALWPDVEPFAEEGLVALSVVNSITCVVPHGARKPLFGTNPIAFAAPCAEHDPIVFDMATSAMAHGDVQIAARAGQQLPEGMGVDADGQPTTDPKAILEGGALLPFGGHKGSALSMMVELLAAALTGGHFSWEFDHSGHPGAETPWTGQLIIVIDPGKAEGQRFAQRSRELVEHMQAVGLTRMPGERRYREREVAEEEGVAVTEQELKGLKELLG

SEQ ID NO: 16 - protein, 332 aa, synthetic construct
MRVPFTELQSLLQAIFQRHGCSEAVARVLAHNCASAQRDGAHSHGVFRMPGYVSTLASGWVDGQATPQVSDVAAGYVRVDAAGGFAQPALAAARELLVAKARSAGIAVLAIHNSHHFAALWPDVEPFAEEGLVALSVVNSVTCVVPHGARKPLFGTNPIAFAAPCAEHDPIVFDMATSAMAHGDVQIAARAGQQLPEGMGVDADGQPTTDPKAILEGGALLPFGGHKGSALSMMVELLAAALTGGHFSWEFDLSGHPGAQTPWTGQLIIVIDPGKAEGQRFAQRSRELVEHMQAVGLTRMPGERRYREREVAEEEGVAVTEQELKGLKELLG

SEQ ID NO: 17 - protein, 332 aa, synthetic construct
MRVPFTELQSLLQAIFQRHGCSEAVARVLAHNCASAQRDGAHSHGVFRMPGYVSTLASGWVDGQATPQVSDVAAGYVRVDAAGGFAQPALAAARELLVAKARSAGIAVLAIHNSHHFAALWPDVEPFAEEGLVALSVVNSVTCVVPHGARKPLFGTNPIAFAAPCAEHDPIVFDMATSAMAHGDVQIAARAGQQLPEGMGVDADGQPTTDPKAILEGGALLPFGGHKGSALSMMVELLAAALTGGHFSWEFDLSGHPGAETPWTGQLIIVIDPGKAEGQRFAQRSRELVEHMQAVGLTRMPGERRYREREVAEEEGVAVTEQELKGLKELLG

SEQ ID NO: 18 - protein, 375 aa, synthetic construct
MRVPFTELQSLLQAIFQRHGCSEAVARVLAHNCASAQRDGAHSHGVFRMPGYVSTLASGWVDGQATPQVSDVAAGYVRVDAAGGFAQPALAAARELLVAKARSAGIAVLAIHNSHHFAALWPDVEPFAEEGLVALSVVNSVTCVVPHGARKPLFGTNPIAFAAPCAEHDPIVFDMATSAMAHGDVQIAARAGQQLPEGMGVDADGQPTTDPKAILEGGALLPFGGHKGSALSMMVELLAAALTGGHFSWEFDQSGHPGAETPWTGQLIIVIDPGKAEGQRFAQRSRELVEHMQAVGLTRMPGERRYREREVAEEEGVAVTEQELKGLKELLGGTDEKTTGWRGGHVVEGLAGELEQLRARLEHHPQGGSHHHHHH

SEQ ID NO: 19 - protein, 375 aa, synthetic construct
MRVPFTELQSLLQAIFQRHGCSEAVARVLAHNCASAQRDGAHSHGVFRMPGYVSTLASGWVDGQATPQVSDVAAGYVRVDAAGGFAQPALAAARELLVAKARSAGIAVLAIHNSHHFAALWPDVEPFAEEGLVALSVVNSITCVVPHGARKPLFGTNPIAFAAPCAEHDPIVFDMATSAMAHGDVQIAARAGQQLPEGMGVDADGQPTTDPKAILEGGALLPFGGHKGSALSMMVELLAAALTGGHFSWEFDHSGHPGAETPWTGQLIIVIDPGKAEGQRFAQRSRELVEHMQAVGLTRMPGERRYREREVAEEEGVAVTEQELKGLKELLGGTDEKTTGWRGGHVVEGLAGELEQLRARLEHHPQGGSHHHHHH

SEQ ID NO: 20 - protein, 375 aa, synthetic construct
MRVPFTELQSLLQAIFQRHGCSEAVARVLAHNCASAQRDGAHSHGVFRMPGYVSTLASGWVDGQATPQVSDVAAGYVRVDAAGGFAQPALAAARELLVAKARSAGIAVLAIHNSHHFAALWPDVEPFAEEGLVALSVVNSVTCVVPHGARKPLFGTNPIAFAAPCAEHDPIVFDMATSAMAHGDVQIAARAGQQLPEGMGVDADGQPTTDPKAILEGGALLPFGGHKGSALSMMVELLAAALTGGHFSWEFDLSGHPGAQTPWTGQLIIVIDPGKAEGQRFAQRSRELVEHMQAVGLTRMPGERRYREREVAEEEGVAVTEQELKGLKELLGGTDEKTTGWRGGHVVEGLAGELEQLRARLEHHPQGGSHHHHHH

SEQ ID NO: 21 - protein, 375 aa, synthetic construct
MRVPFTELQSLLQAIFQRHGCSEAVARVLAHNCASAQRDGAHSHGVFRMPGYVSTLASGWVDGQATPQVSDVAAGYVRVDAAGGFAQPALAAARELLVAKARSAGIAVLAIHNSHHFAALWPDVEPFAEEGLVALSVVNSVTCVVPHGARKPLFGTNPIAFAAPCAEHDPIVFDMATSAMAHGDVQIAARAGQQLPEGMGVDADGQPTTDPKAILEGGALLPFGGHKGSALSMMVELLAAALTGGHFSWEFDLSGHPGAETPWTGQLIIVIDPGKAEGQRFAQRSRELVEHMQAVGLTRMPGERRYREREVAEEEGVAVTEQELKGLKELLGGTDEKTTGWRGGHVVEGLAGELEQLRARLEHHPQGGSHHHHHH